European Patent Specification EP 3 688 030 B1, published December 11, 2024. Title: SPECIFIC BINDING MOLECULES. Applicant: Elasmogen Ltd. The sequence listing filed with the application follows.

SEQUENCE LISTING (96 sequences)

SEQ ID NO: 1 - protein, 11 aa, Artificial Sequence
  TNF VNAR D1 CDR3
ECQYGLAEYDV

SEQ ID NO: 2 - protein, 106 aa, Artificial Sequence
  TNF VNAR D1 CDR3
ARVDQTPQTITKETGESLTINCVLRDSHCATSSTYWYRKKSGSTNEESISKGGRYVETVNSGSKSFSLRINDLTVEDSGTYRCASECQYGLAEYDVYGGGTVVTVN

SEQ ID NO: 3 - protein, 128 aa, Artificial Sequence
  TNF VNAR D1
ARVDQTPQTITKETGESLTINCVLRDSHCATSSTYWYRKKSGSTNEESISKGGRYVETVNSGSKSFSLRINDLTVEDSGTYRCASECQYGLAEYDVYGGGTVVTVNAAAHHHHHHGAAESKLISEEDL

SEQ ID NO: 4 - DNA, 318 bp, Artificial Sequence
  TNF VNAR D1
gctcgagtggaccaaacaccgcaaacaataacaaaggagacgggcgaatcactgaccatcaactgtgtcctacgagatagccactgtgcaacctccagcacgtactggtatcgcaaaaaatcgggctcaacaaacgaggagagcatatcgaaaggtggacgatatgttgaaacagttaacagcggatcaaagtccttttctttgagaattaatgatctaacagttgaagacagtggcacgtatcgatgcgcttccgagtgccaatatggactggcagaatatgatgtatacggaggtggcactgtcgtgactgtgaat

SEQ ID NO: 5 - DNA, 384 bp, Artificial Sequence
  TNF VNAR D1 WITH HIS AND MYC TAGS
gctcgagtggaccaaacaccgcaaacaataacaaaggagacgggcgaatcactgaccatcaactgtgtcctacgagatagccactgtgcaacctccagcacgtactggtatcgcaaaaaatcgggctcaacaaacgaggagagcatatcgaaaggtggacgatatgttgaaacagttaacagcggatcaaagtccttttctttgagaattaatgatctaacagttgaagacagtggcacgtatcgatgcgcttccgagtgccaatatggactggcagaatatgatgtatacggaggtggcactgtcgtgactgtgaatgcggccgcacatcatcatcaccatcacggcgccgcagaatcaaaactcatctcagaagaggatctg

SEQ ID NO: 6 - protein, 14 aa, Artificial Sequence
  TNF VNAR C4 CDR3
SWWTQNWRCSNSDV

SEQ ID NO: 7 - protein, 108 aa, Artificial Sequence
  TNF VNAR C4
RVDQTPQTITKETGESLTINCVLRDSNCGLSSTYWYRKKSGSTNEESISKGGRYVETINEGSKSFSLRINDLTVEDSGTYRCKLSWWTQNWRCSNSDVYGGGTVVTVN

SEQ ID NO: 8 - protein, 131 aa, Artificial Sequence
  TNF VNAR C4 AMINO ACID SEQUENCE WITH HIS AND MYC TAGS
ARVDQTPQTITKETGESLTINCVLRDSNCGLSSTYWYRKKSGSTNEESISKGGRYVETINEGSKSFSLRINDLTVEDSGTYRCKLSWWTQNWRCSNSDVYGGGTVVTVNAAAHHHHHHGAAESKLISEEDL

SEQ ID NO: 9 - DNA, 327 bp, Artificial Sequence
  TNF VNAR C4
gctcgagtggaccaaacaccgcaaacaataacaaaggagacgggcgaatcactgaccatcaactgtgtcctacgagatagcaactgtgggttgtccagcacgtactggtatcgcaaaaaatcgggctcaacaaacgaggagagcatatcgaaaggtggacgatatgttgaaacaattaacgaaggatcaaagtccttttctttgagaattaatgatctaacagttgaagacagtggcacgtatcgatgcaagttaagctggtggacccagaactggagatgctcaaattccgatgtatacggaggtggcactgtcgtgactgtgaat

SEQ ID NO: 10 - DNA, 393 bp, Artificial Sequence
  TNF VNAR D1 WITH HIS AND MYC TAGS
gctcgagtggaccaaacaccgcaaacaataacaaaggagacgggcgaatcactgaccatcaactgtgtcctacgagatagcaactgtgggttgtccagcacgtactggtatcgcaaaaaatcgggctcaacaaacgaggagagcatatcgaaaggtggacgatatgttgaaacaattaacgaaggatcaaagtccttttctttgagaattaatgatctaacagttgaagacagtggcacgtatcgatgcaagttaagctggtggacccagaactggagatgctcaaattccgatgtatacggaggtggcactgtcgtgactgtgaatgcggccgcacatcatcatcaccatcacggcgccgcagaatcaaaactcatctcagaagaggatctg

SEQ ID NO: 11 - protein, 23 aa, Artificial Sequence
  TNF VNAR B4 CDR3
YIPCIDELVYMISGGTSGPIHDV

SEQ ID NO: 12 - protein, 118 aa, Artificial Sequence
  TNF VNAR B4
ARVDQTPQTITKETGESLTINCVLRDSNCALSSMYWYRKKSGSTNEESISKGGRYVETVNSGSKSFSLRINDLTVEDSGTYRCKVYIPCIDELVYMISGGTSGPIHDVYGGGTVVTVN

SEQ ID NO: 13 - protein, 140 aa, Artificial Sequence
  TNF VNAR B4 AMINO ACID SEQUENCE WITH HIS AND MYC TAGS
ARVDQTPQTITKETGESLTINCVLRDSNCALSSMYWYRKKSGSTNEESISKGGRYVETVNSGSKSFSLRINDLTVEDSGTYRCKVYIPCIDELVYMISGGTSGPIHDVYGGGTVVTVNAAAHHHHHHGAAESKLISEEDL

SEQ ID NO: 14 - DNA, 354 bp, Artificial Sequence
  TNF VNAR B4
gctcgagtggaccaaacaccgcaaacaataacaaaggagacgggcgaatcactgaccatcaactgtgtcctacgagatagtaactgtgcattgtccagcatgtactggtatcgcaaaaaatctggctcaacaaacgaggagagcatatcgaaaggtggacgatatgttgaaacagttaacagcggatcaaagtccttttctttgagaattaatgatctaacagttgaagacagtggcacgtatcgatgcaaggtatatataccttgcatcgatgaactggtatatatgatcagtgggggtacctctggcccgattcatgatgtatacggaggtggcactgtcgtgactgtgaat

SEQ ID NO: 15 - DNA, 71 bp, Artificial Sequence
  15
gctaggctctagaaataattttgtttaactttaagaaggagatataccatggctcgagtggaccaaacacc

SEQ ID NO: 16 - DNA, 87 bp, Artificial Sequence
  16
cgcgccggatccgccacctccgctaccgccacctccgctaccgccacctccgctaccgccacctccattcacagtcacgacagtgcc

SEQ ID NO: 17 - DNA, 46 bp, Artificial Sequence
  17
ggtggcggatccggcgcgcactccgctcgagtggaccaaacaccgc

SEQ ID NO: 18 - DNA, 53 bp, Artificial Sequence
  18
gtccggaattctcacagatcctcttctgagatgagtttttgttctgcggcccc

SEQ ID NO: 19 - DNA, 48 bp, Artificial Sequence
  19
aattcccctctagaaggcgcgcactccgctcgagtggaccaaacaccg

SEQ ID NO: 20 - DNA, 420 bp, Artificial Sequence
  TNF VNAR B4 WITH HIS AND MYC TAGS
gctcgagtggaccaaacaccgcaaacaataacaaaggagacgggcgaatcactgaccatcaactgtgtcctacgagatagtaactgtgcattgtccagcatgtactggtatcgcaaaaaatctggctcaacaaacgaggagagcatatcgaaaggtggacgatatgttgaaacagttaacagcggatcaaagtccttttctttgagaattaatgatctaacagttgaagacagtggcacgtatcgatgcaaggtatatataccttgcatcgatgaactggtatatatgatcagtgggggtacctctggcccgattcatgatgtatacggaggtggcactgtcgtgactgtgaatgcggccgcacatcatcatcaccatcacggcgccgcagaatcaaaactcatctcagaagaggatctg

SEQ ID NO: 21 - protein, 249 aa, Artificial Sequence
  TNF VNAR DIMER D1-D1 AMINO ACID SEQUENCE WITH HIS AND MYC TAGS
ARVDQTPQTITKETGESLTINCVLRDSHCATSSTYWYRKKSGSTNEESISKGGRYVETVNSGSKSFSLRINDLTVEDSGTYRCASECQYGLAEYDVYGGGTVVTVNGGGGSGGGGGSGAHSARVDQTPQTITKETGESLTINCVLRDSHCATSSTYWYRKKSGSTNEESISKGGRYVETVNSGSKSFSLRINDLTVEDSGTYRCASECQYGLAEYDVYGGGTVVTVNAAAHHHHHHGAAESKLISEEDL

SEQ ID NO: 22 - DNA, 747 bp, Artificial Sequence
  TNF VNAR DIMER D1-D1 WITH HIS AND MYC TAGS
gctcgagtggaccaaacaccgcaaacaataacaaaggagacgggcgaatcactgaccatcaactgtgtcctacgagatagccactgtgcaacctccagcacgtactggtatcgcaaaaaatcgggctcaacaaacgaggagagcatatcgaaaggtggacgatatgttgaaacagttaacagcggatcaaagtccttttctttgagaattaatgatctaacagttgaagacagtggcacgtatcgatgcgcttccgagtgccaatatggactggcagaatatgatgtatacggaggtggcactgtcgtgactgtgaatggaggtggcggtagcggaggtggtggcggatccggcgcgcactccgctcgagtggaccaaacaccgcaaacaataacaaaggagacgggcgaatcactgaccatcaactgtgtcctacgagatagccactgtgcaacctccagcacgtactggtatcgcaaaaaatcgggctcaacaaacgaggagagcatatcgaaaggtggacgatatgttgaaacagttaacagcggatcaaagtccttttctttgagaattaatgatctaacagttgaagacagtggcacgtatcgatgcgcttccgagtgccaatatggactggcagaatatgatgtatacggaggtggcactgtcgtgactgtgaatgcggccgcacatcatcatcaccatcacggggccgcagaacaaaaactcatctcagaagaggatctg

SEQ ID NO: 23 - protein, 255 aa, Artificial Sequence
  TNF VNAR DIMER C4-C4 AMINO ACID SEQUENCE WITH HIS AND MYC TAGS
ARVDQTPQTITKETGESLTINCVLRDSNCGLSSTYWYRKKSGSTNEESISKGGRYVETINEGSKSFSLRINDLTVEDSGTYRCKLSWWTQNWRCSNSDVYGGGTVVTVNGGGGSGGGGGSGAHSARVDQTPQTITKETGESLTINCVLRDSNCGLSSTYWYRKKSGSTNEESISKGGRYVETINEGSKSFSLRINDLTVEDSGTYRCKLSWWTQNWRCSNSDVYGGGTVVTVNAAAHHHHHHGAAEQKLISEEDL

SEQ ID NO: 24 - DNA, 765 bp, Artificial Sequence
  TNF VNAR DIMER C4-C4 WITH HIS AND MYC TAGS
gctcgagtggaccaaacaccgcaaacaataacaaaggagacgggcgaatcactgaccatcaactgtgtcctacgagatagcaactgtgggttgtccagcacgtactggtatcgcaaaaaatcgggctcaacaaacgaggagagcatatcgaaaggtggacgatatgttgaaacaattaacgaaggatcaaagtccttttctttgagaattaatgatctaacagttgaagacagtggcacgtatcgatgcaagttaagctggtggacccagaactggagatgctcaaattccgatgtatacggaggtggcactgtcgtgactgtgaacggaggtggcggtagcggaggtggtggcggatccggcgcgcactccgctcgagtggaccaaacaccgcaaacaataacaaaggagacgggcgaatcactgaccatcaactgtgtcctacgagatagcaactgtgggttgtccagcacgtactggtatcgcaaaaaatcgggctcaacaaacgaggagagcatatcgaaaggtggacgatatgttgaaacaattaacgaaggatcaaagtccttttctttgagaattaatgatctaacagttgaagacagtggcacgtatcgatgcaagttaagctggtggacccagaactggagatgctcaaattccgatgtatacggaggtggcactgtcgtgactgtgaacgcggccgcacatcatcatcaccatcacggggccgcagaacaaaaactcatctcagaagaggatctg

SEQ ID NO: 25 - protein, 273 aa, Artificial Sequence
  TNF VNAR DIMER B4-B4 AMINO ACID SEQUENCE WITH HIS AND MYC TAGS
ARVDQTPQTITKETGESLTINCVLRDSNCALSSMYWYRKKSGSTNEESISKGGRYVETVNSGSKSFSLRINDLTVEDSGTYRCKVYIPCIDELVYMISGGTSGPIHDVYGGGTVVTVNGGGGSGGGGGSGAHSARVDQTPQTITKETGESLTINCVLRDSNCALSSMYWYRKKSGSTNEESISKGGRYVETVNSGSKSFSLRINDLTVEDSGTYRCKVYIPCIDELVYMISGGTSGPIHDVYGGGTVVTVNAAAHHHHHHGAAEQKLISEEDL

SEQ ID NO: 26 - DNA, 819 bp, Artificial Sequence
  TNF VNAR DIMER B4-B4 WITH HIS AND MYC TAGS
gctcgagtggaccaaacaccgcaaacaataacaaaggagacgggcgaatcactgaccatcaactgtgtcctacgagatagtaactgtgcattgtccagcatgtactggtatcgcaaaaaatctggctcaacaaacgaggagagcatatcgaaaggtggacgatatgttgaaacagttaacagcggatcaaagtccttttctttgagaattaatgatctaacagttgaagacagtggcacgtatcgatgcaaggtatatataccttgcatcgatgaactggtatatatgatcagtgggggtacctctggcccgattcatgatgtatacggaggtggcactgtcgtgactgtgaatggaggtggcggtagcggaggtggtggcggatccggcgcgcactccgctcgagtggaccaaacaccgcaaacaataacaaaggagacgggcgaatcactgaccatcaactgtgtcctacgagatagtaactgtgcattgtccagcatgtactggtatcgcaaaaaatctggctcaacaaacgaggagagcatatcgaaaggtggacgatatgttgaaacagttaacagcggatcaaagtccttttctttgagaattaatgatctaacagttgaagacagtggcacgtatcgatgcaaggtatatataccttgcatcgatgaactggtatatatgatcagtgggggtacctctggcccgattcatgatgtatacggaggtggcactgtcgtgactgtgaatgcggccgcacatcatcatcaccatcacggggccgcagaacaaaaactcatctcagaagaggatctg

SEQ ID NO: 27 - protein, 252 aa, Artificial Sequence
  TNF VNAR DIMER D1-C4 AMINO ACID SEQUENCE WITH HIS AND MYC TAGS
ARVDQTPQTITKETGESLTINCVLRDSHCATSSTYWYRKKSGSTNEESISKGGRYVETVNSGSKSFSLRINDLTVEDSGTYRCASECQYGLAEYDVYGGGTVVTVNGGGGSGGGGGSGAHSARVDQTPQTITKETGESLTINCVLRDSNCGLSSTYWYRKKSGSTNEESISKGGRYVETINEGSKSFSLRINDLTVEDSGTYRCKLSWWTQNWRCSNSDVYGGGTVVTVNAAAHHHHHHGAAEQKLISEEDL

SEQ ID NO: 28 - DNA, 756 bp, Artificial Sequence
  TNF VNAR DIMER D1-C4 WITH HIS AND MYC TAGS
gctcgagtggaccaaacaccgcaaacaataacaaaggagacgggcgaatcactgaccatcaactgtgtcctacgagatagccactgtgcaacctccagcacgtactggtatcgcaaaaaatcgggctcaacaaacgaggagagcatatcgaaaggtggacgatatgttgaaacagttaacagcggatcaaagtccttttctttgagaattaatgatctaacagttgaagacagtggcacgtatcgatgcgcttccgagtgccaatatggactggcagaatatgatgtatacggaggtggcactgtcgtgactgtgaatggaggtggcggtagcggaggtggtggcggatccggcgcgcactccgctcgagtggaccaaacaccgcaaacaataacaaaggagacgggcgaatcactgaccatcaactgtgtcctacgagatagcaactgtgggttgtccagcacgtactggtatcgcaaaaaatcgggctcaacaaacgaggagagcatatcgaaaggtggacgatatgttgaaacaattaacgaaggatcaaagtccttttctttgagaattaatgatctaacagttgaagacagtggcacgtatcgatgcaagttaagctggtggacccagaactggagatgctcaaattccgatgtatacggaggtggcactgtcgtgactgtgaacgcggccgcacatcatcatcaccatcacggggccgcagaacaaaaactcatctcagaagaggatctg

SEQ ID NO: 29 - protein, 261 aa, Artificial Sequence
  TNF VNAR DIMER D1-B4 AMINO ACID SEQUENCE WITH HIS AND MYC TAGS
ARVDQTPQTITKETGESLPINCVLRDSHCATSSTYWYRKKSGSTNEESISKGGRYVETVNSGSKSFSLRINDLTVEDSGTYRCASECQYGLAEYDVYGGGTVVTVNGGGGSGGGGGSGAHSARVDQTPQTITKETGESLTINCVLRDSNCALSSMYWYRKKSGSTNEESISKGGRYVETVNSGSKSFSLRINDLTVEDSGTYRCKVYIPCIDELVYMISGGTSGPIHDVYGGGTVVTVNAAAHHHHHHGAAEQKLISEEDL

SEQ ID NO: 30 - DNA, 783 bp, Artificial Sequence
  NUCLEOTIDE SEQUENCE CODIGN FOR THE TNF VNAR DIMER D1-B4 NUCLEOTIDE SEQUENCE WITH HIS AND MYC TAGS
gctcgagtggaccaaacaccgcaaacaataacaaaggagacgggcgaatcactgaccatcaactgtgtcctacgagatagccactgtgcaacctccagcacgtactggtatcgcaaaaaatcgggctcaacaaacgaggagagcatatcgaaaggtggacgatatgttgaaacagttaacagcggatcaaagtccttttctttgagaattaatgatctaacagttgaagacagtggcacgtatcgatgcgcttccgagtgccaatatggactggcagaatatgatgtatacggaggtggcactgtcgtgactgtgaatggaggtggcggtagcggaggtggtggcggatccggcgcgcactccgctcgagtggaccaaacaccgcaaacaataacaaaggagacgggcgaatcactgaccatcaactgtgtcctacgagatagtaactgtgcattgtccagcatgtactggtatcgcaaaaaatctggctcaacaaacgaggagagcatatcgaaaggtggacgatatgttgaaacagttaacagcggatcaaagtccttttctttgagaattaatgatctaacagttgaagacagtggcacgtatcgatgcaaggtatatataccttgcatcgatgaactggtatatatgatcagtgggggtacctctggcccgattcatgatgtatacggaggtggcactgtcgtgactgtgaatgcggccgcacatcatcatcaccatcacggggccgcagaacaaaaactcatctcagaagaggatctg

SEQ ID NO: 31 - protein, 261 aa, Artificial Sequence
  TNF VNAR DIMER B4-D1 AMINO ACID SEQUENCE
ARVDQTPQTITKETGESLTINCVLRDSNCALSSMYWYRKKSGSTNEESISKGGRYVETVNSGSKSFSLRINDLTVEDSGTYRCKVYIPCIDELVYMISGGTSGPIHDVYGGGTVVTVNGGGGSGGGGGSGAHSARVDQTPQTITKETGESLPINCVLRDSHCATSSTYWYRKKSGSTNEESISKGGRYVETVNSGSKSFSLRINDLTVEDSGTYRCASECQYGLAEYDVYGGGTVVTVNAAAHHHHHHGAAEQKLISEEDL

SEQ ID NO: 32 - DNA, 783 bp, Artificial Sequence
  TNF VNAR DIMER B4-D1 NUCLEOTIDE SEQUENCE
gctcgagtggaccaaacaccgcaaacaataacaaaggagacgggcgaatcactgaccatcaactgtgtcctacgagatagtaactgtgcattgtccagcatgtactggtatcgcaaaaaatctggctcaacaaacgaggagagcatatcgaaaggtggacgatatgttgaaacagttaacagcggatcaaagtccttttctttgagaattaatgatctaacagttgaagacagtggcacgtatcgatgcaaggtatatataccttgcatcgatgaactggtatatatgatcagtgggggtacctctggcccgattcatgatgtatacggaggtggcactgtcgtgactgtgaatggaggtggcggtagcggaggtggtggcggatccggcgcgcactccgctcgagtggaccaaacaccgcaaacaataacaaaggagacgggcgaatcactgaccatcaactgtgtcctacgagatagccactgtgcaacctccagcacgtactggtatcgcaaaaaatcgggctcaacaaacgaggagagcatatcgaaaggtggacgatatgttgaaacagttaacagcggatcaaagtccttttctttgagaattaatgatctaacagttgaagacagtggcacgtatcgatgcgcttccgagtgccaatatggactggcagaatatgatgtatacggaggtggcactgtcgtgactgtgaatgcggccgcacatcatcatcaccatcacggggccgcagaacaaaaactcatctcagaagaggatctg

SEQ ID NO: 33 - protein, 263 aa, Artificial Sequence
  TNF VNAR DIMER C4-B4 AMINO ACID SEQUENCE
ARVDQTPQTITKETGESLTINCVLRDSNCGLSSTYWYRKKSGSTNEESISKGGRYVETINEGSKSFSLRINDLTVEDSGTYRCKLSWWTQNWRCSNSDVYGGGTVVTVNGGGGSGGGGGSGAHSARVDQTPQTITKETGESLTINCVLRDSNCALSSMYWYRKKSGSTNEESISKGGRYVETVNSGSKSFSLRINDLTVEDSGTYRCKVYIPCIDELVYMISGGTSGPIHDVYGGGTVVTVNAAAHHHHHHGAAEQKLISEED

SEQ ID NO: 34 - DNA, 792 bp, Artificial Sequence
  TNF VNAR DIMER C4-B4 NUCLEOTIDE SEQUENCE
gctcgagtggaccaaacaccgcaaacaataacaaaggagacgggcgaatcactgaccatcaactgtgtcctacgagatagcaactgtgggttgtccagcacgtactggtatcgcaaaaaatcgggctcaacaaacgaggagagcatatcgaaaggtggacgatatgttgaaacaattaacgaaggatcaaagtccttttctttgagaattaatgatctaacagttgaagacagtggcacgtatcgatgcaagttaagctggtggacccagaactggagatgctcaaattccgatgtatacggaggtggcactgtcgtgactgtgaacggaggtggcggtagcggaggtggtggcggatccggcgcgcactccgctcgagtggaccaaacaccgcaaacaataacaaaggagacgggcgaatcactgaccatcaactgtgtcctacgagatagtaactgtgcattgtccagcatgtactggtatcgcaaaaaatctggctcaacaaacgaggagagcatatcgaaaggtggacgatatgttgaaacagttaacagcggatcaaagtccttttctttgagaattaatgatctaacagttgaagacagtggcacgtatcgatgcaaggtatatataccttgcatcgatgaactggtatatatgatcagtgggggtacctctggcccgattcatgatgtatacggaggtggcactgtcgtgactgtgaatgcggccgcacatcatcatcaccatcacggggccgcagaacaaaaactcatctcagaagaggatctg

SEQ ID NO: 35 - protein, 263 aa, Artificial Sequence
  TNF VNAR DIMER B4-C4 AMINO ACID SEQUENCE
ARVDQTPQTITKETGESLTINCVLRDSNCALSSMYWYRKKSGSTNEESISKGGRYVETVNSGSKSFSLRINDLTVEDSGTYRCKVYIPCIDELVYMISGGTSGPIHDVYGGGTVVTVNGGGGSGGGGGSGAHSARVDQTPQTITKETGESLTINCVLRDSNCGLSSTYWYRKKSGSTNEESISKGGRYVETINEGSKSFSLRINDLTVEDSGTYRCKLSWWTQNWRCSNSDVYGGGTVVTVNAAAHHHHHHGAAEQKLISEED

SEQ ID NO: 36 - DNA, 792 bp, Artificial Sequence
  TNF VNAR DIMER B4-C4 NUCLEOTIDE SEQUENCE
gctcgagtggaccaaacaccgcaaacaataacaaaggagacgggcgaatcactgaccatcaactgtgtcctacgagatagtaactgtgcattgtccagcatgtactggtatcgcaaaaaatctggctcaacaaacgaggagagcatatcgaaaggtggacgatatgttgaaacagttaacagcggatcaaagtccttttctttgagaattaatgatctaacagttgaagacagtggcacgtatcgatgcaaggtatatataccttgcatcgatgaactggtatatatgatcagtgggggtacctctggcccgattcatgatgtatacggaggtggcactgtcgtgactgtgaatggaggtggcggtagcggaggtggtggcggatccggcgcgcactccgctcgagtggaccaaacaccgcaaacaataacaaaggagacgggcgaatcactgaccatcaactgtgtcctacgagatagcaactgtgggttgtccagcacgtactggtatcgcaaaaaatcgggctcaacaaacgaggagagcatatcgaaaggtggacgatatgttgaaacaattaacgaaggatcaaagtccttttctttgagaattaatgatctaacagttgaagacagtggcacgtatcgatgcaagttaagctggtggacccagaactggagatgctcaaattccgatgtatacggaggtggcactgtcgtgactgtgaacgcggccgcacatcatcatcaccatcacggggccgcagaacaaaaactcatctcagaagaggatctg

SEQ ID NO: 37 - protein, 383 aa, Artificial Sequence
  TNF VNAR D1-BA11-C4 AMINO ACID SEQUENCE WITH HIS AND MYC TAGS
ARVDQTPQTITKETGESLTINCVLRDSHCATSSTYWYRKKSGSTNEESISKGGRYVETVNSGSKSFSLRINDLTVEDSGTYRCASECQYGLAEYDVYGGGTVVTVNGGGGSGGGGSGGGGSGGGGSGAHSTRVDQSPSSLSASVGDRVTITCVLTDTSYPLYSTYWYRKNPGSSNKEQISISGRYSESVNKGTKSFTLTISSLQPEDSATYYCRAMSTNIWTGDGAGTKVEIKGGGGSGGGGSGGGGSGGGGSGAHSARVDQTPQTITKETGESLTINCVLRDSNCGLSSTYWYRKKSGSTNEESISKGGRYVETINEGSKSFSLRINDLTVEDSGTYRCKLSWWTQNWRCSNSDVYGGGTVVTVNHHHHHHHEQKLISEEDL

SEQ ID NO: 38 - DNA, 1149 bp, Artificial Sequence
  NUCLEOTIDE SEQUENCE CODING FOR THE TNF VNAR D1-BA11-C4 WITH HIS AND MYC TAGS
gctcgagtggaccaaacaccgcaaacaataacaaaggagacgggcgaatcactgaccatcaactgtgtcctacgagatagccactgtgcaacctccagcacgtactggtatcgcaaaaaatcgggctcaacaaacgaggagagcatatcgaaaggtggacgatatgttgaaacagttaacagcggatcaaagtccttttctttgagaattaatgatctaacagttgaagacagtggcacgtatcgatgcgcttccgagtgccaatatggactggcagaatatgatgtatacggaggtggcactgtcgtgactgtgaatggaggtggcggatccgggggtggcggtagcggaggtggcggtagcggaggtggcggtagtggagctcattcaacaagagtggaccaaagtccaagctctctgtccgccagtgtgggcgaccgcgtgaccatcacctgcgtcctgactgataccagctatcctctgtacagcacatactggtatcggaagaatcccggttccagcaacaaggagcagatttccatctccggccgctatagtgaatcagtcaacaagggcactaagtcctttaccctgacaatcagttccctgcagcccgaggactccgccacctattactgcagagctatgagtacaaatatctggaccggggacggagctggtaccaaggtggagatcaagggaggtggcggttccggaggtggcggtagcggaggtggcggtagcggaggtggcggtagcggggcccattctgctcgagtggaccaaacaccgcaaacaataacaaaggagacgggcgaatcactgaccatcaactgtgtcctacgagatagcaactgtgggttgtccagcacgtactggtatcgcaaaaaatcgggctcaacaaacgaggagagcatatcgaaaggtggacgatatgttgaaacaattaacgaaggatcaaagtccttttctttgagaattaatgatctaacagttgaagacagtggcacgtatcgatgcaagttaagctggtggacccagaactggagatgctcaaattccgatgtatacggaggtggcactgtcgtgactgtgaatcatcaccatcaccatcaccatgaacaaaaactcatctcagaagaggatctg

SEQ ID NO: 39 - protein, 380 aa, Artificial Sequence
  TNF VNAR D1-BA11-D1 AMINO ACID SEQUENCE WITH HIS AND MYC TAGS
ARVDQTPQTITKETGESLTINCVLRDSHCATSSTYWYRKKSGSTNEESISKGGRYVETVNSGSKSFSLRINDLTVEDSGTYRCASECQYGLAEYDVYGGGTVVTVNGGGGSGGGGSGGGGSGGGGSGAHSTRVDQSPSSLSASVGDRVTITCVLTDTSYPLYSTYWYRKNPGSSNKEQISISGRYSESVNKGTKSFTLTISSLQPEDSATYYCRAMSTNIWTGDGAGTKVEIKGGGGSGGGGSGGGGSGGGGSGAHSARVDQTPQTITKETGESLTINCVLRDSHCATSSTYWYRKKSGSTNEESISKGGRYVETVNSGSKSFSLRINDLTVEDSGTYRCASECQYGLAEYDVYGGGTVVTVNHHHHHHHEQKLISEEDL

SEQ ID NO: 40 - DNA, 1140 bp, Artificial Sequence
  NUCLEOTIDE SEQUENCE CODING FOR THE TNF VNAR D1-BA11-D1 WITH HIS AND MYC TAGS
gctcgagtggaccaaacaccgcaaacaataacaaaggagacgggcgaatcactgaccatcaactgtgtcctacgagatagccactgtgcaacctccagcacgtactggtatcgcaaaaaatcgggctcaacaaacgaggagagcatatcgaaaggtggacgatatgttgaaacagttaacagcggatcaaagtccttttctttgagaattaatgatctaacagttgaagacagtggcacgtatcgatgcgcttccgagtgccaatatggactggcagaatatgatgtatacggaggtggcactgtcgtgactgtgaatggaggtggcggatccgggggtggcggtagcggaggtggcggtagcggaggtggcggtagtggagctcattcaacaagagtggaccaaagtccaagctctctgtccgccagtgtgggcgaccgcgtgaccatcacctgcgtcctgactgataccagctatcctctgtacagcacatactggtatcggaagaatcccggttccagcaacaaggagcagatttccatctccggccgctatagtgaatcagtcaacaagggcactaagtcctttaccctgacaatcagttccctgcagcccgaggactccgccacctattactgcagagctatgagtacaaatatctggaccggggacggagctggtaccaaggtggagatcaagggaggtggcggttccggaggtggcggtagcggaggtggcggtagcggaggtggcggtagcggggcccattctgctcgagtggaccaaacaccgcaaacaataacaaaggagacgggcgaatcactgaccatcaactgtgtcctacgagatagccactgtgcaacctccagcacgtactggtatcgcaaaaaatcgggctcaacaaacgaggagagcatatcgaaaggtggacgatatgttgaaacagttaacagcggatcaaagtccttttctttgagaattaatgatctaacagttgaagacagtggcacgtatcgatgcgcttccgagtgccaatatggactggcagaatatgatgtatacggaggtggcactgtcgtgactgtgaatcatcaccatcaccatcaccatgaacaaaaactcatctcagaagaggatctg

SEQ ID NO: 41 - protein, 392 aa, Artificial Sequence
  TNF VNAR D1-BA11-B4 AMINO ACID SEQUENCE WITH HIS AND MYC TAGS
ARVDQTPQTITKETGESLTINCVLRDSHCATSSTYWYRKKSGSTNEESISKGGRYVETVNSGSKSFSLRINDLTVEDSGTYRCASECQYGLAEYDVYGGGTVVTVNGGGGSGGGGSGGGGSGGGGSGAHSTRVDQSPSSLSASVGDRVTITCVLTDTSYPLYSTYWYRKNPGSSNKEQISISGRYSESVNKGTKSFTLTISSLQPEDSATYYCRAMSTNIWTGDGAGTKVEIKGGGGSGGGGSGGGGSGGGGSGAHSARVDQTPQTITKETGESLTINCVLRDSNCALSSMYWYRKKSGSTNEESISKGGRYVETVNSGSKSFSLRINDLTVEDSGTYRCKVYIPCIDELVYMISGGTSGPIHDVYGGGTVVTVNHHHHHHHEQKLISEEDL

SEQ ID NO: 42 - DNA, 1176 bp, Artificial Sequence
  NUCLEOTIDE SEQUENCE CODING FOR THE TNF VNAR D1-BA11-B4 WITH HIS AND MYC TAGS
gctcgagtggaccaaacaccgcaaacaataacaaaggagacgggcgaatcactgaccatcaactgtgtcctacgagatagccactgtgcaacctccagcacgtactggtatcgcaaaaaatcgggctcaacaaacgaggagagcatatcgaaaggtggacgatatgttgaaacagttaacagcggatcaaagtccttttctttgagaattaatgatctaacagttgaagacagtggcacgtatcgatgcgcttccgagtgccaatatggactggcagaatatgatgtatacggaggtggcactgtcgtgactgtgaatggaggtggcggatccgggggtggcggtagcggaggtggcggtagcggaggtggcggtagtggagctcattcaacaagagtggaccaaagtccaagctctctgtccgccagtgtgggcgaccgcgtgaccatcacctgcgtcctgactgataccagctatcctctgtacagcacatactggtatcggaagaatcccggttccagcaacaaggagcagatttccatctccggccgctatagtgaatcagtcaacaagggcactaagtcctttaccctgacaatcagttccctgcagcccgaggactccgccacctattactgcagagctatgagtacaaatatctggaccggggacggagctggtaccaaggtggagatcaagggaggtggcggttccggaggtggcggtagcggaggtggcggtagcggaggtggcggtagcggggcccattctgctcgagtggaccaaacaccgcaaacaataacaaaggagacgggcgaatcactgaccatcaactgtgtcctacgagatagtaactgtgcattgtccagcatgtactggtatcgcaaaaaatctggctcaacaaacgaggagagcatatcgaaaggtggacgatatgttgaaacagttaacagcggatcaaagtccttttctttgagaattaatgatctaacagttgaagacagtggcacgtatcgatgcaaggtatatataccttgcatcgatgaactggtatatatgatcagtgggggtacctctggcccgattcatgatgtatacggaggtggcactgtcgtgactgtgaatcatcaccatcaccatcaccatgaacaaaaactcatctcagaagaggatctg

SEQ ID NO: 43 - protein, 485 aa, Artificial Sequence
  ICOS VNAR 2D4-Fc-2D4 AMINO ACID SEQUENCE
TRVDQTPRTATKETGESLTINCVLTDTDYGLFSTSWFRKNPGTTDWERMSIGGRYVESVNKGAKSFSLRIKDLTVADSATYYCKAFTWPWEWPDRWFRPWYDGAGTVLTVNGGGGSGGGADQEPKSSDKTHTCPPCPAPELLGGPSVFLFPPKPKDTLMISRTPEVTCVVVDVSHEDPEVKFNWYVDGVEVHNAKTKPREEQYNSTYRVVSVLTVLHQDWLNGKEYKCKVSNKALPAPIEKTISKAKGQPREPQVYTLPPSREEMTKNQVSLTCLVKGFYPSDIAVEWESNGQPENNYKTTPPVLDSDGSFFLYSKLTVDKSRWQQGNVFSCSVMHEALHNHYTQKSLSLSPGKTAAAATAAAATAAAATAAAATRVDQTPRTATKETGESLTINCVLTDTDYGLFSTSWFRKNPGTTDWERMSIGGRYVESVNKGAKSFSLRIKDLTVADSATYYCKAFTWPWEWPDRWFRPWYDGAGTVLTVN

SEQ ID NO: 44 - DNA, 1455 bp, Artificial Sequence
  ICOS VNAR 2D4-Fc-2D4
acacgtgttgaccagacaccgcgtaccgcaaccaaagaaaccggtgaaagcctgaccattaattgtgttctgaccgataccgattatggtttgttctccaccagctggtttcgtaaaaatccgggtacaaccgattgggaacgtatgagcattggtggtcgttatgttgaaagcgtgaataaaggtgccaaaagctttagcctgcgcattaaagatctgaccgttgcagatagcgcaacctattactgtaaagcattcacttggccgtgggaatggccggaccgttggttccgtccgtggtatgatggtgcaggcaccgttctgaccgttaatggcggtggtggttctggtggtggtgctgatcaggagcccaaatcttctgacaaaactcacacatgtccaccgtgcccagcacctgaactcctgggtggaccgtcagtcttcctcttccccccaaaacccaaggacaccctcatgatctcccggacccctgaggtcacatgcgtggtggtggacgtgagccacgaagaccctgaggtcaagttcaactggtacgtggacggcgtggaggtgcataatgccaagacaaagccgcgggaggagcagtacaacagcacgtaccgtgtggtcagcgtcctcaccgtcctgcaccaggactggctgaatggcaaggagtacaagtgcaaggtctccaacaaagccctcccagcccccatcgagaaaaccatctccaaagccaaagggcagccccgagaaccacaggtgtacaccctgcccccatcccgggaggagatgaccaagaaccaggtcagcctgacctgcctggtcaaaggcttctatcccagcgacatcgccgtggagtgggagagcaatgggcagccggagaacaactacaagaccacgcctcccgtgctggactccgacggctccttcttcctctatagcaagctcaccgtggacaagagcaggtggcagcaggggaacgtcttctcatgctccgtgatgcatgaggctctgcacaaccactacacgcagaagagcctctccctgtccccgggtaaaaccgccgccgccgccaccgccgccgccgccaccgccgccgccgccaccgccgcggccgccacacgtgttgatcagacaccgcgtaccgcaaccaaagaaaccggtgaaagcctgaccattaattgtgttctgaccgataccgattatggtttgttctccaccagctggtttcgtaaaaatccgggtacaaccgattgggaacgtatgagcattggtggtcgttatgttgaaagcgtgaataaaggtgccaaaagctttagcctgcgcattaaagatctgaccgttgcagatagcgcaacctattactgtaaagcattcacttggccgtgggaatggccggaccgttggttccgtccgtggtatgatggtgcaggcaccgttctgaccgttaat

SEQ ID NO: 45 - protein, 481 aa, Artificial Sequence
  ICOS VNAR 2D4-Fc-CC3 AMINO ACID SEQUENCE
TRVDQTPRTATKETGESLTINCVLTDTDYGLFSTSWFRKNPGTTDWERMSIGGRYVESVNKGAKSFSLRIKDLTVADSATYYCKAFTWPWEWPDRWFRPWYDGAGTVLTVNGGGGSGGGADQEPKSSDKTHTCPPCPAPELLGGPSVFLFPPKPKDTLMISRTPEVTCVVVDVSHEDPEVKFNWYVDGVEVHNAKTKPREEQYNSTYRVVSVLTVLHQDWLNGKEYKCKVSNKALPAPIEKTISKAKGQPREPQVYTLPPSREEMTKNQVSLTCLVKGFYPSDIAVEWESNGQPENNYKTTPPVLDSDGSFFLYSKLTVDKSRWQQGNVFSCSVMHEALHNHYTQKSLSLSPGKTAAAATAAAATAAAATAAAATRVDQTPRTATKETGESLTINCVLTDTEYGLFSTSWFRKNPGTTDWERMSIGGRYVESVNKGAKSFSLRIKDLTVADSATYYCKALGWWPPAFPHWYDGAGTVLTVN

SEQ ID NO: 46 - DNA, 1443 bp, Artificial Sequence
  ICOS VNAR 2D4-Fc-CC3
acacgtgttgaccagacaccgcgtaccgcaaccaaagaaaccggtgaaagcctgaccattaattgtgttctgaccgataccgattatggtttgttctccaccagctggtttcgtaaaaatccgggtacaaccgattgggaacgtatgagcattggtggtcgttatgttgaaagcgtgaataaaggtgccaaaagctttagcctgcgcattaaagatctgaccgttgcagatagcgcaacctattactgtaaagcattcacttggccgtgggaatggccggaccgttggttccgtccgtggtatgatggtgcaggcaccgttctgaccgttaatggcggtggtggttctggtggtggtgctgatcaggagcccaaatcttctgacaaaactcacacatgtccaccgtgcccagcacctgaactcctgggtggaccgtcagtcttcctcttccccccaaaacccaaggacaccctcatgatctcccggacccctgaggtcacatgcgtggtggtggacgtgagccacgaagaccctgaggtcaagttcaactggtacgtggacggcgtggaggtgcataatgccaagacaaagccgcgggaggagcagtacaacagcacgtaccgtgtggtcagcgtcctcaccgtcctgcaccaggactggctgaatggcaaggagtacaagtgcaaggtctccaacaaagccctcccagcccccatcgagaaaaccatctccaaagccaaagggcagccccgagaaccacaggtgtacaccctgcccccatcccgggaggagatgaccaagaaccaggtcagcctgacctgcctggtcaaaggcttctatcccagcgacatcgccgtggagtgggagagcaatgggcagccggagaacaactacaagaccacgcctcccgtgctggactccgacggctccttcttcctctatagcaagctcaccgtggacaagagcaggtggcagcaggggaacgtcttctcatgctccgtgatgcatgaggctctgcacaaccactacacgcagaagagcctctccctgtccccgggtaaaaccgccgccgccgccaccgccgccgccgccaccgccgccgccgccaccgccgcggccgccacacgtgttgatcagacaccgcgtaccgcaaccaaagaaaccggtgaaagcctgaccattaattgtgttctgaccgataccgagtatggtttgttctccaccagctggtttcgtaaaaatccgggtacaaccgattgggaacgtatgagcattggtggtcgttatgttgaaagcgtgaataaaggtgccaaaagctttagcctgcgcattaaagatctgaccgttgcagatagcgcaacctattactgtaaagcactgggttggtggccgccggctttcccgcattggtatgatggtgcaggcaccgttctgaccgttaat

SEQ ID NO: 47 - protein, 481 aa, Artificial Sequence
  ICOS VNAR CC3-Fc-2D4 AMINO ACID SEQUENCE
TRVDQTPRTATKETGESLTINCVLTDTEYGLFSTSWFRKNPGTTDWERMSIGGRYVESVNKGAKSFSLRIKDLTVADSATYYCKALGWWPPAFPHWYDGAGTVLTVNGGGGSGGGGRTEPKSSDKTHTCPPCPAPEAAGAPSVFLFPPKPKDTLMISRTPEVTCVVVDVSHEDPEVKFNWYVDGVEVHNAKTKPREEQYNSTYRVVSVLTVLHQDWLNGKEYKCKVSNKALPAPIEKTISKAKGQPREPQVYTLPPSREEMTKNQVSLTCLVKGFYPSDIAVEWESNGQPENNYKTTPPVLDSDGSFFLYSKLTVDKSRWQQGNVFSCSVMHEALHNHYTQKSLSLSPGKTAAAATAAAATAAAATAAAATRVDQTPRTATKETGESLTINCVLTDTDYGLFSTSWFRKNPGTTDWERMSIGGRYVESVNKGAKSFSLRIKDLTVADSATYYCKAFTWPWEWPDRWFRPWYDGAGTVLTVN

SEQ ID NO: 48 - DNA, 1443 bp, Artificial Sequence
  ICOS VNAR CC3-Fc-2D4
acacgtgttgatcagacaccgcgtaccgcaaccaaagaaaccggtgaaagcctgaccattaattgtgttctgaccgataccgagtatggtttgttctccaccagctggtttcgtaaaaatccgggtacaaccgattgggaacgtatgagcattggtggtcgttatgttgaaagcgtgaataaaggtgccaaaagctttagcctgcgcattaaagatctgaccgttgcagatagcgcaacctattactgtaaagcactgggttggtggccgccggctttcccgcattggtatgatggtgcaggcaccgttctgaccgttaatggcggtggtggttctggtggtggtggtcgtacggagcccaaatcttctgacaaaactcacacatgcccaccgtgcccagcacctgaagccgctggggcaccgtcagtcttcctcttccccccaaaacccaaggacaccctcatgatctcccggacccctgaggtcacatgcgtggtggtggacgtgagccacgaagaccctgaggtcaagttcaactggtacgtggacggcgtggaggtgcataatgccaagacaaagccgcgggaggagcagtacaacagcacgtaccgtgtggtcagcgtcctcaccgtcctgcaccaggactggctgaatggcaaggagtacaagtgcaaggtctccaacaaagccctcccagcccccatcgagaaaaccatctccaaagccaaagggcagccccgagaaccacaggtgtacaccctgcccccatcccgggaggagatgaccaagaaccaggtcagcctgacctgcctggtcaaaggcttctatcccagcgacatcgccgtggagtgggagagcaatgggcagccggagaacaactacaagaccacgcctcccgtgctggactccgacggctccttcttcctctatagcaagctcaccgtggacaagagcaggtggcagcaggggaacgtcttctcatgctccgtgatgcatgaggctctgcacaaccactacacgcagaagagcctctccctgtccccgggtaaaaccgccgccgccgccaccgccgccgccgccaccgccgccgccgccaccgccgcggccgccacacgtgttgatcagacaccgcgtaccgcaaccaaagaaaccggtgaaagcctgaccattaattgtgttctgaccgataccgattatggtttgttctccaccagctggtttcgtaaaaatccgggtacaaccgattgggaacgtatgagcattggtggtcgttatgttgaaagcgtgaataaaggtgccaaaagctttagcctgcgcattaaagatctgaccgttgcagatagcgcaacctattactgtaaagcattcacttggccgtgggaatggccggaccgttggttccgtccgtggtatgatggtgcaggcaccgttctgaccgttaat

SEQ ID NO: 49 - protein, 477 aa, Artificial Sequence
  ICOS VNAR CC3-Fc-CC3 AMINO ACID SEQUENCE
TRVDQTPRTATKETGESLTINCVLTDTEYGLFSTSWFRKNPGTTDWERMSIGGRYVESVNKGAKSFSLRIKDLTVADSATYYCKALGWWPPAFPHWYDGAGTVLTVNGGGGSGGGGRTEPKSSDKTHTCPPCPAPEAAGAPSVFLFPPKPKDTLMISRTPEVTCVVVDVSHEDPEVKFNWYVDGVEVHNAKTKPREEQYNSTYRVVSVLTVLHQDWLNGKEYKCKVSNKALPAPIEKTISKAKGQPREPQVYTLPPSREEMTKNQVSLTCLVKGFYPSDIAVEWESNGQPENNYKTTPPVLDSDGSFFLYSKLTVDKSRWQQGNVFSCSVMHEALHNHYTQKSLSLSPGKTAAAATAAAATAAAATAAAATRVDQTPRTATKETGESLTINCVLTDTEYGLFSTSWFRKNPGTTDWERMSIGGRYVESVNKGAKSFSLRIKDLTVADSATYYCKALGWWPPAFPHWYDGAGTVLTVN

SEQ ID NO: 50 - DNA, 1431 bp, Artificial Sequence
  ICOS VNAR CC3-Fc-CC3
acacgtgttgatcagacaccgcgtaccgcaaccaaagaaaccggtgaaagcctgaccattaattgtgttctgaccgataccgagtatggtttgttctccaccagctggtttcgtaaaaatccgggtacaaccgattgggaacgtatgagcattggtggtcgttatgttgaaagcgtgaataaaggtgccaaaagctttagcctgcgcattaaagatctgaccgttgcagatagcgcaacctattactgtaaagcactgggttggtggccgccggctttcccgcattggtatgatggtgcaggcaccgttctgaccgttaatggcggtggtggttctggtggtggtggtcgtacggagcccaaatcttctgacaaaactcacacatgcccaccgtgcccagcacctgaagccgctggggcaccgtcagtcttcctcttccccccaaaacccaaggacaccctcatgatctcccggacccctgaggtcacatgcgtggtggtggacgtgagccacgaagaccctgaggtcaagttcaactggtacgtggacggcgtggaggtgcataatgccaagacaaagccgcgggaggagcagtacaacagcacgtaccgtgtggtcagcgtcctcaccgtcctgcaccaggactggctgaatggcaaggagtacaagtgcaaggtctccaacaaagccctcccagcccccatcgagaaaaccatctccaaagccaaagggcagccccgagaaccacaggtgtacaccctgcccccatcccgggaggagatgaccaagaaccaggtcagcctgacctgcctggtcaaaggcttctatcccagcgacatcgccgtggagtgggagagcaatgggcagccggagaacaactacaagaccacgcctcccgtgctggactccgacggctccttcttcctctatagcaagctcaccgtggacaagagcaggtggcagcaggggaacgtcttctcatgctccgtgatgcatgaggctctgcacaaccactacacgcagaagagcctctccctgtccccgggtaaaaccgccgccgccgccaccgccgccgccgccaccgccgccgccgccaccgccgcggccgccacacgtgttgatcagacaccgcgtaccgcaaccaaagaaaccggtgaaagcctgaccattaattgtgttctgaccgataccgagtatggtttgttctccaccagctggtttcgtaaaaatccgggtacaaccgattgggaacgtatgagcattggtggtcgttatgttgaaagcgtgaataaaggtgccaaaagctttagcctgcgcattaaagatctgaccgttgcagatagcgcaacctattactgtaaagcactgggttggtggccgccggctttcccgcattggtatgatggtgcaggcaccgttctgaccgttaat

SEQ ID NO: 51 - protein, 112 aa, Artificial Sequence
  SoloMER  VNAR D1-v1 AMINO ACID SEQUENCE WITH HIS TAG
ARVDQSPSSLSASVGDRVTITCVLRDSHCATSSTYWYRKKSGSTNEESISKGGRYVETVNSGSKSFSLRINDLTVEDSGTYRCASECQYGLAEYDVYGGGTKVEIKHHHHHH

SEQ ID NO: 52 - DNA, 336 bp, Artificial Sequence
  NUCLEOTIDE SEQUENCE CODING FOR THE SoloMER  VNAR D1-v1 WITH HIS TAG
gcccgcgtggaccagtccccctcctccctgtccgcctccgtgggcgaccgcgtgaccatcacctgcgtgctgcgcgactcccactgcgccacctcctccacctactggtaccgcaagaagtccggctccaccaacgaggagtccatctccaaggggggccgctacgtggagaccgtgaactccggctccaagtccttctccctgcgcatcaacgacctgaccgtggaggactccggcacctaccgctgcgcctccgagtgccagtacggcctggccgagtacgacgtgtacggcggcggcaccaaggtggagatcaagcaccaccaccaccaccac

SEQ ID NO: 53 - protein, 112 aa, Artificial Sequence
  SoloMER  VNAR D1-v2 AMINO ACID SEQUENCE WITH HIS TAG
ARVDQSPSSLSASVGDRVTITCVLRDSHCATSSTYWYRKKSGSTNEESISKGGRYVETVNSGSKSFTLTISSLQPEDFATYYCASECQYGLAEYDVYGGGTKVEIKHHHHHH

SEQ ID NO: 54 - DNA, 336 bp, Artificial Sequence
  NUCLEOTIDE SEQUENCE CODING FOR THE SoloMER  VNAR D1-v2 WITH HIS TAG
gcccgcgtggaccagtccccctcctccctgtccgcctccgtgggcgaccgcgtgaccatcacctgcgtgctgcgcgactcccactgcgccacctcctccacctactggtaccgcaagaagtccggctccaccaacgaggagtccatctccaaggggggccgctacgtggagaccgtgaactccggctccaagtccttcaccctgaccatctcctccctgcagcccgaggacttcgccacctactactgcgcctccgagtgccagtacggcctggccgagtacgacgtgtacggcggcggcaccaaggtggagatcaagcaccaccaccaccaccac

SEQ ID NO: 55 - protein, 112 aa, Artificial Sequence
  SoloMER  VNAR D1-v3 AMINO ACID SEQUENCE WITH HIS TAG
ARVDQSPSSLSASVGDRVTITCVLRDSHCATSSTYWYQQKPGKTNEESISKGGRYVETVNSGSKSFTLTISSLQPEDFATYYCASECQYGLAEYDVYGGGTKVEIKHHHHHH

SEQ ID NO: 56 - DNA, 336 bp, Artificial Sequence
  NUCLEOTIDE SEQUENCE CODING FOR THE SoloMER  VNAR D1-v3 WITH HIS TAG
gcccgcgtggaccagtccccctcctccctgtccgcctccgtgggcgaccgcgtgaccatcacctgcgtgctgcgcgactcccactgcgccacctcctccacctactggtaccagcagaagcccggcaagaccaacgaggagtccatctccaaggggggccgctacgtggagaccgtgaactccggctccaagtccttcaccctgaccatctcctccctgcagcccgaggacttcgccacctactactgcgcctccgagtgccagtacggcctggccgagtacgacgtgtacggcggcggcaccaaggtggagatcaagcaccaccaccaccaccac

SEQ ID NO: 57 - protein, 112 aa, Artificial Sequence
  SoloMER  VNAR D1-v4 AMINO ACID SEQUENCE WITH HIS TAG
ARVDQSPSSLSASVGDRVTITCVLRDSHCATSSTYWYRKKPGSTNEESISKGGRFSGSGSSGSKSFTLTISSLQPEDFATYYCASECQYGLAEYDVFGQGTKVEIKHHHHHH

SEQ ID NO: 58 - DNA, 336 bp, Artificial Sequence
  NUCLEOTIDE SEQUENCE CODING FOR THE SoloMER  VNAR D1-v4 WITH HIS TAG
gcccgcgtggaccagtccccctcctccctgtccgcctccgtgggcgaccgcgtgaccatcacctgcgtgctgcgcgactcccactgcgccacctcctccacctactggtaccgcaagaagcccggctccaccaacgaggagtccatctccaaggggggccgcttctccggctccggctcctccggctccaagtccttcaccctgaccatctcctccctgcagcccgaggacttcgccacctactactgcgcctccgagtgccagtacggcctggccgagtacgacgtgttcggccagggcaccaaggtggagatcaagcaccaccaccaccaccac

SEQ ID NO: 59 - protein, 483 aa, Artificial Sequence
  Quad-X  D1-Fc-C4 AMINO ACID SEQUENCE
ARVDQTPQTITKETGESLTINCVLRDSHCATSSTYWYRKKSGSTNEESISKGGRYVETVNSGSKSFSLRINDLTVEDSGTYRCASECQYGLAEYDVYGGGTVVTVNGSGGGSGGGGSGEPKSSDKTHTCPPCPAPELLGGPSVFLFPPKPKDTLMISRTPEVTCVVVDVSHEDPEVKFNWYVDGVEVHNAKTKPREEQYNSTYRVVSVLTVLHQDWLNGKEYKCKVSNKALPAPIEKTISKAKGQPREPQVYTLPPSRDELTKNQVSLTCLVKGFYPSDIAVEWESNGQPENNYKTTPPVLDSDGSFFLYSKLTVDKSRWQQGNVFSCSVMHEALHNHYTQKSLSLSPGKGGGGSGGGGSGGGGSGGGGSGAHSARVDQTPQTITKETGESLTINCVLRDSNCGLSSTYWYRKKSGSTNEESISKGGRYVETINEGSKSFSLRINDLTVEDSGTYRCKLSWWTQNWRCSNSDVYGGGTVVTVN

SEQ ID NO: 60 - DNA, 1449 bp, Artificial Sequence
  NUCLEOTIDE SEQUENCE CODING FOR THE Quad-X  D1-Fc-C4
gctcgagtggaccaaacaccgcaaacaataacaaaggagacgggcgaatcactgaccatcaactgtgtcctacgagatagccactgtgcaacctccagcacgtactggtatcgcaaaaaatcgggctcaacaaacgaggagagcatatcgaaaggtggacgatatgttgaaacagttaacagcggatcaaagtccttttctttgagaattaatgatctaacagttgaagacagtggcacgtatcgatgcgcttccgagtgccaatatggactggcagaatatgatgtatacggaggtggcactgtcgtgactgtgaatggatccggtggtgggtccggaggaggtggctcaggagagcccaaatctagcgacaaaactcacacatgcccaccgtgcccagcacctgaactcctggggggaccgtcagtcttcctcttccccccaaaacccaaggacaccctcatgatctcccggacccctgaggtcacatgcgtggtggtggacgtgagccacgaagaccctgaggtcaagttcaactggtacgtggacggcgtggaggtgcataatgccaagacaaagccgcgggaggagcagtacaacagcacgtaccgggtggtcagcgtcctcaccgtcctgcaccaggactggctgaatggcaaggagtacaagtgcaaggtctccaacaaagccctcccagcccccatcgagaaaaccatctccaaagccaaagggcagccccgagaaccacaggtgtacaccctgcccccatcccgggatgagctgaccaagaaccaggtcagcctgacctgcctggtcaaaggcttctatcccagcgacatcgccgtggagtgggagagcaatgggcagccggagaacaactacaagaccacgcctcccgtgctggactccgacggctccttcttcctctacagcaagctcaccgtggacaagagcaggtggcagcaggggaacgtcttctcatgctccgtgatgcatgaggctctgcacaaccactacacgcagaagagcctctccctgtctccggggaaaggaggtggcggttccggaggtggcggtagcggaggtggcggtagcggaggtggcggtagcggggcccattctgctcgagtggaccaaacaccgcaaacaataacaaaggagacgggcgaatcactgaccatcaactgtgtcctacgagatagcaactgtgggttgtccagcacgtactggtatcgcaaaaaatcgggctcaacaaacgaggagagcatatcgaaaggtggacgatatgttgaaacaattaacgaaggatcaaagtccttttctttgagaattaatgatctaacagttgaagacagtggcacgtatcgatgcaagttaagctggtggacccagaactggagatgctcaaattccgatgtatacggaggtggcactgtcgtgactgtgaat

SEQ ID NO: 61 - protein, 472 aa, Artificial Sequence
  Quad-Y-D1C4  D1-C4-Fc AMINO ACID SEQUENCE
ARVDQTPQTITKETGESLTINCVLRDSHCATSSTYWYRKKSGSTNEESISKGGRYVETVNSGSKSFSLRINDLTVEDSGTYRCASECQYGLAEYDVYGGGTVVTVNGGGGSGGGGGSGAHSARVDQTPQTITKETGESLTINCVLRDSNCGLSSTYWYRKKSGSTNEESISKGGRYVETINEGSKSFSLRINDLTVEDSGTYRCKLSWWTQNWRCSNSDVYGGGTVVTVNGGGSGGGGSGEPKSSDKTHTCPPCPAPELLGGPSVFLFPPKPKDTLMISRTPEVTCVVVDVSHEDPEVKFNWYVDGVEVHNAKTKPREEQYNSTYRVVSVLTVLHQDWLNGKEYKCKVSNKALPAPIEKTISKAKGQPREPQVYTLPPSRDELTKNQVSLTCLVKGFYPSDIAVEWESNGQPENNYKTTPPVLDSDGSFFLYSKLTVDKSRWQQGNVFSCSVMHEALHNHYTQKSLSLSPGK

SEQ ID NO: 62 - DNA, 1416 bp, Artificial Sequence
  NUCLEOTIDE SEQUENCE CODING FOR THE Quad-Y-D1C4  AMINO ACID SEQUENCE
gctcgagtggaccaaacaccgcaaacaataacaaaggagacgggcgaatcactgaccatcaactgtgtcctacgagatagccactgtgcaacctccagcacgtactggtatcgcaaaaaatcgggctcaacaaacgaggagagcatatcgaaaggtggacgatatgttgaaacagttaacagcggatcaaagtccttttctttgagaattaatgatctaacagttgaagacagtggcacgtatcgatgcgcttccgagtgccaatatggactggcagaatatgatgtatacggaggtggcactgtcgtgactgtgaatggaggtggcggtagcggaggtggtggcggatccggggcgcactccgctcgagtggaccaaacaccgcaaacaataacaaaggagacgggcgaatcactgaccatcaactgtgtcctacgagatagcaactgtgggttgtccagcacgtactggtatcgcaaaaaatcgggctcaacaaacgaggagagcatatcgaaaggtggacgatatgttgaaacaattaacgaaggatcaaagtccttttctttgagaattaatgatctaacagttgaagacagtggcacgtatcgatgcaagttaagctggtggacccagaactggagatgctcaaattccgatgtatacggaggtggcactgtcgtgactgtgaacggtggtgggtccggaggaggtggctcaggagagcccaaatctagcgacaaaactcacacatgcccaccgtgcccagcacctgaactcctggggggaccgtcagtcttcctcttccccccaaaacccaaggacaccctcatgatctcccggacccctgaggtcacatgcgtggtggtggacgtgagccacgaagaccctgaggtcaagttcaactggtacgtggacggcgtggaggtgcataatgccaagacaaagccgcgggaggagcagtacaacagcacgtaccgtgtggtcagcgtcctcaccgtcctgcaccaggactggctgaatggcaaggagtacaagtgcaaggtctccaacaaagccctcccagcccccatcgagaaaaccatctccaaagccaaagggcagccccgagaaccacaggtgtacaccctgcccccatcccgggatgagctgaccaagaaccaggtcagcctgacctgcctggtcaaaggcttctatcccagcgacatcgccgtggagtgggagagcaatgggcagccggagaacaactacaagaccacgcctcccgtgctggactccgacggctccttcttcctctacagcaagctcaccgtggacaagagcaggtggcagcaggggaacgtcttctcatgctccgtgatgcatgaggctctgcacaaccactacacgcagaagagcctctccctgtctccggggaaa

SEQ ID NO: 63 - protein, 472 aa, Artificial Sequence
  Quad-Y-C4D1  C4-D1-Fc AMINO ACID SEQUENCE
ARVDQTPQTITKETGESLTINCVLRDSNCGLSSTYWYRKKSGSTNEESISKGGRYVETINEGSKSFSLRINDLTVEDSGTYRCKLSWWTQNWRCSNSDVYGGGTVVTVNGGGGSGGGGGSGAHSARVDQTPQTITKETGESLTINCVLRDSHCATSSTYWYRKKSGSTNEESISKGGRYVETVNSGSKSFSLRINDLTVEDSGTYRCASECQYGLAEYDVYGGGTVVTVNGGGSGGGGSGEPKSSDKTHTCPPCPAPELLGGPSVFLFPPKPKDTLMISRTPEVTCVVVDVSHEDPEVKFNWYVDGVEVHNAKTKPREEQYNSTYRVVSVLTVLHQDWLNGKEYKCKVSNKALPAPIEKTISKAKGQPREPQVYTLPPSRDELTKNQVSLTCLVKGFYPSDIAVEWESNGQPENNYKTTPPVLDSDGSFFLYSKLTVDKSRWQQGNVFSCSVMHEALHNHYTQKSLSLSPGK

SEQ ID NO: 64 - protein, 1416 aa, Artificial Sequence
  NUCLEOTIDE SEQUENCE CODING FOR THE Quad-Y-C4D1  AMINO ACID SEQUENCE
GCTCGAGTGGACCAAACACCGCAAACAATAACAAAGGAGACGGGCGAATCACTGACCATCAACTGTGTCCTACGAGATAGCAACTGTGGGTTGTCCAGCACGTACTGGTATCGCAAAAAATCGGGCTCAACAAACGAGGAGAGCATATCGAAAGGTGGACGATATGTTGAAACAATTAACGAAGGATCAAAGTCCTTTTCTTTGAGAATTAATGATCTAACAGTTGAAGACAGTGGCACGTATCGATGCAAGTTAAGCTGGTGGACCCAGAACTGGAGATGCTCAAATTCCGATGTATACGGAGGTGGCACTGTCGTGACTGTGAACGGAGGTGGCGGTAGCGGAGGTGGTGGCGGATCCGGGGCGCACTCCGCTCGAGTGGACCAAACACCGCAAACAATAACAAAGGAGACGGGCGAATCACTGACCATCAACTGTGTCCTACGAGATAGCCACTGTGCAACCTCCAGCACGTACTGGTATCGCAAAAAATCGGGCTCAACAAACGAGGAGAGCATATCGAAAGGTGGACGATATGTTGAAACAGTTAACAGCGGATCAAAGTCCTTTTCTTTGAGAATTAATGATCTAACAGTTGAAGACAGTGGCACGTATCGATGCGCTTCCGAGTGCCAATATGGACTGGCAGAATATGATGTATACGGAGGTGGCACTGTCGTGACTGTGAATGGTGGTGGGTCCGGAGGAGGTGGCTCAGGAGAGCCCAAATCTAGCGACAAAACTCACACATGCCCACCGTGCCCAGCACCTGAACTCCTGGGGGGACCGTCAGTCTTCCTCTTCCCCCCAAAACCCAAGGACACCCTCATGATCTCCCGGACCCCTGAGGTCACATGCGTGGTGGTGGACGTGAGCCACGAAGACCCTGAGGTCAAGTTCAACTGGTACGTGGACGGCGTGGAGGTGCATAATGCCAAGACAAAGCCGCGGGAGGAGCAGTACAACAGCACGTACCGTGTGGTCAGCGTCCTCACCGTCCTGCACCAGGACTGGCTGAATGGCAAGGAGTACAAGTGCAAGGTCTCCAACAAAGCCCTCCCAGCCCCCATCGAGAAAACCATCTCCAAAGCCAAAGGGCAGCCCCGAGAACCACAGGTGTACACCCTGCCCCCATCCCGGGATGAGCTGACCAAGAACCAGGTCAGCCTGACCTGCCTGGTCAAAGGCTTCTATCCCAGCGACATCGCCGTGGAGTGGGAGAGCAATGGGCAGCCGGAGAACAACTACAAGACCACGCCTCCCGTGCTGGACTCCGACGGCTCCTTCTTCCTCTACAGCAAGCTCACCGTGGACAAGAGCAGGTGGCAGCAGGGGAACGTCTTCTCATGCTCCGTGATGCATGAGGCTCTGCACAACCACTACACGCAGAAGAGCCTCTCCCTGTCTCCGGGGAAA

SEQ ID NO: 65 - protein, 111 aa, Artificial Sequence
  2D4
TRVDQTPRTATKETGESLTINCVLTDTDYGLFSTSWFRKNPGTTDWERMSIGGRYVESVNKGAKSFSLRIKDLTVADSATYYCKAFTWPWEWPDRWFRPWYDGAGTVLTVN

SEQ ID NO: 66 - protein, 107 aa, Artificial Sequence
  CC3
TRVDQTPRTATKETGESLTINCVLTDTEYGLFSTSWFRKNPGTTDWERMSIGGRYVESVNKGAKSFSLRIKDLTVADSATYYCKALGWWPPAFPHWYDGAGTVLTVN

SEQ ID NO: 67 - protein, 103 aa, Artificial Sequence
  BA11
TRVDQSPSSLSASVGDRVTITCVLTDTSYPLYSTYWYRKNPGSSNKEQISISGRYSESVNKGTKSFTLTISSLQPEDSATYYCRAMSTNIWTGDGAGTKVEIK

SEQ ID NO: 68 - protein, 6 aa, Artificial Sequence
  TNF-alpha specific VNAR binding domain CDR1
HCATSS

SEQ ID NO: 69 - protein, 6 aa, Artificial Sequence
  TNF-alpha spcific VNAR binding domain CDR1
NCGLSS

SEQ ID NO: 70 - protein, 6 aa, Artificial Sequence
  TNF-alpha specific VNAR binding domain CDR1
NCALSS

SEQ ID NO: 71 - protein, 9 aa, Artificial Sequence
  TNF-alpha specific VNAR binding domain hyper-variable region 2
TNEESISKG

SEQ ID NO: 72 - protein, 5 aa, Artificial Sequence
  TNF-alpha specific VNAR binding domain hyper-variable region 4
SGSKS

SEQ ID NO: 73 - protein, 5 aa, Artificial Sequence
  TNF-alpha specific VNAR binding domain hyper-variable region 4
EGSKS

SEQ ID NO: 74 - DNA, 46 bp, Artificial Sequence
  NARF4For1 primer
ataatcaagcttgcggccgcattcacagtcacgacagtgccacctc

SEQ ID NO: 75 - DNA, 46 bp, Artificial Sequence
  NARF4For2 primer
ataatcaagcttgcggccgcattcacagtcacggcagtgccatctc

SEQ ID NO: 76 - DNA, 39 bp, Artificial Sequence
  NARF1Rev primer
ataataaggaattccatggctcgagtggaccaaacaccg

SEQ ID NO: 77 - protein, 103 aa, Artificial Sequence
  E06
TRVDQTPRTATRETGESLTINCVLTDTSYPLYSTYWYRKNPGSSNKEQISISGRYVESVNKGTKSFSLRIKDLTVADSATYICRAMGTNIWTGDGAGTVLTVN

SEQ ID NO: 78 - protein, 103 aa, Artificial Sequence
  hE06v1.10
TRVDQSPSSLSASVGDRVTITCVLTDTSYPLYSTYWYRKNPGSSNKEQISISGRYSESVNKGTKSFTLTISSLQPEDFATYYCRAMGTNIWTGDGAGTKVEIK

SEQ ID NO: 79 - protein, 103 aa, Artificial Sequence
  AC9
TRVDQSPSSLSASVGDRVTITCVLTDTSYPLYSTYWYRKNPGSSNKEQISISGRYSESVNKGTKSSTLTISSLQPEDFATYYCRAMGTNIWTGDGAGTKVEIK

SEQ ID NO: 80 - protein, 103 aa, Artificial Sequence
  AD4
TRVDQSPSSLSASVGDRVTITCVLTDTSYPLYSTYWYRKNPGSSNKEQISMSGRYSESVNKSTKSFTLTISSLQPEDFATYYCRAMGTNIWTGDGAGTKVEIK

SEQ ID NO: 81 - protein, 103 aa, Artificial Sequence
  AG11
TRVDQSPSSLSASVGDRVTITCVLTDTSYPLYSTYWYRKNPGSSNKEQISISGRYSESVNKGTKSFTLTISSLQPEDFATYYCRAMGTNIWTGDGAGTKVETK

SEQ ID NO: 82 - protein, 103 aa, Artificial Sequence
  AH7
TRVDQTPSSLSASVGDRVTITCVLTDTSYPLYSTYWYRKNPGSSNKEQISISGRYSESVNKGTKSSTLTISSLQPEDFATYYCRAMGTNIWTGDGAGTKVEIK

SEQ ID NO: 83 - protein, 103 aa, Artificial Sequence
  BB10
TRVDQSPSSLSASVGDRVTITCVLTDTSYPLYSTYWYRKNPGSSNKEQISISGRYSESVNKGTKSFTLTISSLQPEDFATYYCRAMGTNFWTGDGAGTKVEIK

SEQ ID NO: 84 - protein, 103 aa, Artificial Sequence
  BB11
TRVDQSPSSLSASVGDRVTITCVLTDTSYPLYSTYWYRKNPGSSNKEQISISGRYSESVNKGTKSFTLTISSLQPEDFATYYCRAMATNIWTGDGAGTKVEIK

SEQ ID NO: 85 - protein, 103 aa, Artificial Sequence
  BC3
TRVDQSPSSLSASVGDRVTITCVLTDTSYPLYSTYWYRKNPGSNNKEQISISGRYSESVNKGTKSFTLTISSLQPEDFATYYCRAMGTNIWTGDGAGTKVEIK

SEQ ID NO: 86 - protein, 103 aa, Artificial Sequence
  BD12
TRVDQSPSSLSASVGDRVTITCVLTDTSYPLYSTYWYRKNPGSSNKEQISISGRYSESVNKGTNSFTLTISSLQPEDFATYYCRAMGTNIWTGDGAGTKVEIK

SEQ ID NO: 87 - protein, 103 aa, Artificial Sequence
  BE4
TRVDQSPSSLSASVGDRVTITCVLTDTSYSLYSTYWYRKNPGSSNKEQISISGRYSESVNKGTKSFTLTISSLQPEDFATYYCRAMGTNIWTGDGAGTKVEIK

SEQ ID NO: 88 - protein, 103 aa, Artificial Sequence
  BH4
TRVDQSPSSLSASVGDRVTITCVLTDTSYPLYSTYWYRKNPGSSNKEQISISGRYSESVNKGTKSFTLTISSLQPEDFATYYCRAMGTNLWTGDGAGTKVEIK

SEQ ID NO: 89 - protein, 239 aa, Artificial Sequence
  Artificial Sequence
ARVDQTPQTITKETGESLTINCVLRDSHCATSSTYWYRKKSGSTNEESISKGGRYVETVNSGSKSFSLRINDLTVEDSGTYRCASECQYGLAEYDVYGGGTVVTVNGGGGSGGGGGSGGGSARVDQTPQTITKETGESLTINCVLRDSNCGLSSTYWYRKKSGSTNEESISKGGRYVETINEGSKSFSLRINDLTVEDSGTYRCKLSWWTQNWRCSNSDVYGGGTVVTVNAAAHHHHHH

SEQ ID NO: 90 - DNA, 717 bp, Artificial Sequence
  Artificial Sequence
gctcgagtggaccaaacaccgcaaacaataacaaaggagacgggcgaatcactgaccatcaactgtgtcctacgagatagccactgtgcaacctccagcacgtactggtatcgcaaaaaatcgggctcaacaaacgaggagagcatatcgaaaggtggacgatatgttgaaacagttaacagcggatcaaagtccttttctttgagaattaatgatctaacagttgaagacagtggcacgtatcgatgcgcttccgagtgccaatatggactggcagaatatgatgtatacggaggtggcactgtcgtgactgtgaatggaggtggcggtagcggaggtggtggcggatccggcggtggttccgctcgagtggaccaaacaccgcaaacaataacaaaggagacgggcgaatcactgaccatcaactgtgtcctacgagatagcaactgtgggttgtccagcacgtactggtatcgcaaaaaatcgggctcaacaaacgaggagagcatatcgaaaggtggacgatatgttgaaacaattaacgaaggatcaaagtccttttctttgagaattaatgatctaacagttgaagacagtggcacgtatcgatgcaagttaagctggtggacccagaactggagatgctcaaattccgatgtatacggaggtggcactgtcgtgactgtgaacgcggccgcacatcatcatcaccatcac

SEQ ID NO: 91 - protein, 239 aa, Artificial Sequence
  Artificial Sequence
ARVDQSPSSLSASVGDRVTITCVLRDSHCATSSTYWYRKKSGSTNEESISKGGRYVETVNSGSKSFTLTISSLQPEDFATYYCASECQYGLAEYDVYGGGTKVEIKGGGGSGGGGGSGGGSARVDQSPSSLSASVGDRVTITCVLRDSNCGLSSTYWYRKKSGSTNEESISKGGRYVETINEGSKSFSLRINDLTVEDSGTYRCKLSWWTQNWRCSNSDVYGGGTKVEIKAAAHHHHHH

SEQ ID NO: 92 - DNA, 717 bp, Artificial Sequence
  Artificial Sequence
gcccgcgtggaccagtccccctcctccctgtccgcctccgtgggcgaccgcgtgaccatcacctgcgtgctgcgcgactcccactgcgccacctcctccacctactggtaccgcaagaagtccggctccaccaacgaggagtccatctccaaggggggccgctacgtggagaccgtgaactccggctccaagtccttcaccctgaccatctcctccctgcagcccgaggacttcgccacctactactgcgcctccgagtgccagtacggcctggccgagtacgacgtgtacggcggcggcaccaaggtggagatcaagggaggtggcggtagcggaggtggtggcggatccggcggtggttccgcccgcgtggaccagtccccctcctccctgtccgcctccgtgggcgaccgcgtgaccatcacctgcgtgctgcgcgactccaactgcggcctgtcctccacctactggtaccgcaagaagtccggctccaccaacgaggagtccatctccaagggcggccgctacgtggagaccatcaacgagggctccaagtccttctccctgcgcatcaacgacctgaccgtggaggactccggcacctaccgctgcaagctgtcctggtggacccagaactggcgctgctccaactccgacgtgtacggcggcggcaccaaggtggagatcaaggcggccgcacatcatcatcaccatcac

SEQ ID NO: 93 - protein, 249 aa, Artificial Sequence
  Artificial Sequence
ARVDQSPSSLSASVGDRVTITCVLRDSHCATSSTYWYRKKSGSTNEESISKGGRYVETVNSGSKSFTLTISSLQPEDFATYYCASECQYGLAEYDVYGGGTKVEIKGGGGSGGGGSGGGGSGGGGSGGGGSARVDQSPSSLSASVGDRVTITCVLRDSNCGLSSTYWYRKKSGSTNEESISKGGRYVETINEGSKSFSLRINDLTVEDSGTYRCKLSWWTQNWRCSNSDVYGGGTKVEIKAAAHHHHHH

SEQ ID NO: 94 - DNA, 747 bp, Artificial Sequence
  Artificial Sequence
gcccgcgtggaccagtccccctcctccctgtccgcctccgtgggcgaccgcgtgaccatcacctgcgtgctgcgcgactcccactgcgccacctcctccacctactggtaccgcaagaagtccggctccaccaacgaggagtccatctccaaggggggccgctacgtggagaccgtgaactccggctccaagtccttcaccctgaccatctcctccctgcagcccgaggacttcgccacctactactgcgcctccgagtgccagtacggcctggccgagtacgacgtgtacggcggcggcaccaaggtggagatcaagggtggtggtggtagcggtggtggcggttcaggtggcggtggttctggcggtggcggtagtggcggaggtggtagtgcccgcgtggaccagtccccctcctccctgtccgcctccgtgggcgaccgcgtgaccatcacctgcgtgctgcgcgactccaactgcggcctgtcctccacctactggtaccgcaagaagtccggctccaccaacgaggagtccatctccaagggcggccgctacgtggagaccatcaacgagggctccaagtccttctccctgcgcatcaacgacctgaccgtggaggactccggcacctaccgctgcaagctgtcctggtggacccagaactggcgctgctccaactccgacgtgtacggcggcggcaccaaggtggagatcaaggcggccgcacatcatcatcaccatcac

SEQ ID NO: 95 - protein, 484 aa, Artificial Sequence
  Artificial Sequence
ASVNQTPRTATKETGESLTINCVLTDTHAKVFTTSWFRKNPGTTDWERMSIGGRYVESVNKGAKSFSLRIKDLTVADSATYICRAGGYLSQPRVYWDVYGAGTVLTVNGGGGSGGGGRTEPRGPTIKPCPPCKCPAPNLLGGPSVFIFPPKIKDVLMISLSPIVTCVVVDVSEDDPDVQISWFVNNVEVHTAQTQTHREDYNSTLRVVSALPIQHQDWMSGKEFKCKVNNKDLPAPIERTISKPKGSVRAPQVYVLPPPEEEMTKKQVTLTCMVTDFMPEDIYVEWTNNGKTELNYKNTEPVLDSDGSYFMYSKLRVEKKNWVERNSYSCSVVHEGLHNHHTTKSFSRTPGKGGGGSGGGGSGGGGSGGGGSGAHSASVNQTPRTATKETGESLTINCVLTDTHAKVFTTSWFRKNPGTTDWERMSIGGRYVESVNKGAKSFSLRIKDLTVADSATYICRAGGYLSQPRVYWDVYGAGTVLTVN

SEQ ID NO: 96 - DNA, 1452 bp, Artificial Sequence
  Artificial Sequence
gcaagcgttaatcagacaccgcgtaccgcaaccaaagaaaccggtgaaagcctgaccattaattgtgttctgaccgatacccatgctaaagttttcactaccagctggtttcgtaaaaatccgggtacaaccgattgggaacgtatgagcattggtggtcgttatgttgaaagcgtgaataaaggtgccaaaagctttagcctgcgcattaaagatctgaccgttgcagatagcgcaacctatatctgtcgtgccggtggttacctgtctcagccgcgtgtttactgggatgtttatggtgcaggcaccgttctgaccgttaatggcggtggtggttctggtggtggtggtcgtacggagcctcgaggccccacaatcaagccctgtcctccatgcaaatgcccagcacctaacctcttgggtggaccatccgtcttcatcttccctccaaagatcaaggatgtactcatgatctccctgagccccatagtcacatgtgtggtggtggatgtgagcgaggatgacccagatgtccagatcagctggtttgtgaacaacgtggaagtacacacagctcagacacaaacccatagagaggattacaacagtactctccgggtggtcagtgccctccccatccagcaccaggactggatgagtggcaaggagttcaaatgcaaggtcaacaacaaagacctcccagcgcccatcgagagaaccatctcaaaacccaaagggtcagtaagagctccacaggtatatgtcttgcctccaccagaagaagagatgactaagaaacaggtcactctgacctgcatggtcacagacttcatgcctgaagacatttacgtggagtggaccaacaacgggaaaacagagctaaactacaagaacactgaaccagtcctggactctgatggttcttacttcatgtacagcaagctgagagtggaaaagaagaactgggtggaaagaaatagctactcctgttcagtggtccacgagggtctgcacaatcaccacacgactaagagcttctcccggactccgggtaaaggaggtggcggttccggaggtggcggtagcggaggtggcggtagcggaggtggcggtagcggggcccattctgcaagcgttaatcagacaccgcgtaccgcaaccaaagaaaccggtgaaagcctgaccattaattgtgttctgaccgatacccatgctaaagttttcactaccagctggtttcgtaaaaatccgggtacaaccgattgggaacgtatgagcattggtggtcgttatgttgaaagcgtgaataaaggtgccaaaagctttagcctgcgcattaaagatctgaccgttgcagatagcgcaacctatatctgtcgtgccggtggttacctgtctcagccgcgtgtttactgggatgtttatggtgcaggcaccgttctgaccgttaat